European Patent Specification EP 3 854 888 B1, published April 16, 2025. Title: composition for identification of Lactobacilus acidophilus strain and method of determination thereof. Applicant: KOREA FOOD RESEARCH INSTITUTE. The sequence listing filed with the application follows.

SEQUENCE LISTING (21 sequences)

SEQ ID NO: 1 - DNA, 24 bp, Artificial Sequence
  CRISPR_LA_uni_F
taaaagctacagagttaccatcga

SEQ ID NO: 2 - DNA, 25 bp, Artificial Sequence
  CRISPR_LA_uni_S1-S4_F
ggctctaaaagctacagagttacca

SEQ ID NO: 3 - DNA, 25 bp, Artificial Sequence
  CRISPR_LA_uni_S1-S3_F
ggctctaaaagctacagagttacca

SEQ ID NO: 4 - DNA, 24 bp, Artificial Sequence
  CRISPR_LA_uni_S2-S5_F
tcatcgtaagaaataagtcgcata

SEQ ID NO: 5 - DNA, 26 bp, Artificial Sequence
  CRISPR_LA_uni_S2-S4_F
tctcatcgtaagaaataagtcgcata

SEQ ID NO: 6 - DNA, 24 bp, Artificial Sequence
  CRISPR_LA_uni_S3-S5_F
ccttttcctaggatcttcataagc

SEQ ID NO: 7 - DNA, 20 bp, Artificial Sequence
  CRISPR_YT1_F
ttgacttgcgctaggtgttg

SEQ ID NO: 8 - DNA, 20 bp, Artificial Sequence
  CRISPR_LA_F
ttgacttgcgctaggtgttg

SEQ ID NO: 9 - DNA, 20 bp, Artificial Sequence
  CRISPR_LA_uni_R
attgatgcaacacctagcgc

SEQ ID NO: 10 - DNA, 22 bp, Artificial Sequence
  CRISPR_LA_uni_S1-S4_R
cagggtggttttaagtacgaga

SEQ ID NO: 11 - DNA, 20 bp, Artificial Sequence
  CRISPR_LA_uni_S1-S3_R
tggcgagaagcttatgaaga

SEQ ID NO: 12 - DNA, 20 bp, Artificial Sequence
  CRISPR_LA_uni_S2-S5_R
caacacctagcgcaagtcaa

SEQ ID NO: 13 - DNA, 22 bp, Artificial Sequence
  CRISPR_LA_uni_S2-S4_R
cagggtggttttaagtacgaga

SEQ ID NO: 14 - DNA, 21 bp, Artificial Sequence
  CRISPR_LA_uni_S3-S5_R
atgcaacacctagcgcaagtc

SEQ ID NO: 15 - DNA, 20 bp, Artificial Sequence
  CRISPR_YT1_R
tcaccagaaagcgttgttcc

SEQ ID NO: 16 - DNA, 20 bp, Artificial Sequence
  CRISPR_LA_R
gcgtggcaaatgaatggttg

SEQ ID NO: 17 - DNA, 267 bp, Artificial Sequence
  amplicon sequence
taaaagctacagagttaccatcgaggatcacctccactttcgtggagaaaattggaatctcatcgtaagaaataagtcgcatataggatcacctccacatacgtggagaaaatccttttcctaggatcttcataagcttctcgccaggatcacctccacatacgtggagaaaatatcgtagtcaatctcgtacttaaaaccaccctgggatcacctccacatacgtggagaaaatccaggttgacttgcgctaggtgttgcatcaat

SEQ ID NO: 18 - DNA, 897 bp, Artificial Sequence
  amplicon sequence
catcaataggatcacctccacatacgtggagaaaattaggcaaatagccaatttttatcatacattccgggatcacctccacatacgtggagaaaatcggcaatttttgaaacaaacaactatgtatataggatcacctccacatacgtggagaaaataaataaggaagatattgccaccctcggtacccaggatcacctccacatacgtggagaaaatacaagttttgctctaaccatgatgttgtaaacaggatcacctccacatacgtggagaaaatacgttaaagcggacaataagcttcaacgttttaggatcacctccacatacgtggagaaaatcgtgcttgaaattgctctcggggtttcgcctaaggatcacctccacatacgtggagaaaatatttgctgcgagtaactctgacttgtttacccgggatcacctccacatacgtggagaaaattttagctaagtttaagaccgaagatggccaaagggatcacctccacatacgtggagaaaatcggcaatttttgaaacaaacaactatgtatataggatcacctccacatacgtggagaaaatcggcaatttttgaaacaaacaactatgtatataggatcacctccacatacgtggagaaaatacaagttttgctctaaccatgatgttgtaaacaggatcacctccacatacgtggagaaaatagctatccaaatattaaatttgcactagttaaggggatcacctccacatacgtggagaaaatgaagaattttatcttctaggtggcttttttgtgggatcacctccacatacgtggagaaaatagaaatatttgattttgatagtgaaaaagaataggatcacctccacatacgtggagaaattcagtcc

SEQ ID NO: 19 - DNA, 837 bp, Artificial Sequence
  amplicon sequence
catcaataggatcacctccacatacgtggagaaaattaggcaaatagccaatttttatcatacattccgggatcacctccacatacgtggagaaaatcggcaatttttgaaacaaacaactatgtatataggatcacctccacatacgtggagaaaataaataaggaagatattgccaccctcggtacccaggatcacctccacatacgtggagaaaatacgttaaagcggacaataagcttcaacgttttaggatcacctccacatacgtggagaaaatcgtgcttgaaattgctctcggggtttcgcctaaggatcacctccacatacgtggagaaaatatttgctgcgagtaactctgacttgtttacccgggatcacctccacatacgtggagaaaattttagctaagtttaagaccgaagatggccaaagggatcacctccacatacgtggagaaaatcggcaatttttgaaacaaacaactatgtatataggatcacctccacatacgtggagaaaatcggcaatttttgaaacaaacaactatgtatataggatcacctccacatacgtggagaaaatacaagttttgctctaaccatgatgttgtaaacaggatcacctccacatacgtggagaaaatagctatccaaatattaaatttgcactagttaaggggatcacctccacatacgtggagaaaatgaagaattttatcttctaggtggcttttttgtgggatcacctccacatacgtggagaaaatagaaatatttgattttgatagtgaaaaagaataggatcacctccacatacgtggagaaattcagatac

SEQ ID NO: 20 - DNA, 165 bp, Artificial Sequence
  amplicon sequence
catcaataggatcacctccacatacgtggagaaaatgaagaattttatcttctaggtggcttttttgtgggatcacctccacatacgtggagaaaatagaaatatttgattttgatagtgaaaaagaataggatcacctccacatacgtggagaaaattcaagat

SEQ ID NO: 21 - DNA, 320 bp, Artificial Sequence
  amplicon sequence
ttgacttgcgctaggtgttgcatcaataggatcacctccacatacgtggagaaaatgacaccaaaaagggcggtggaaaacttttcaaaggatcacctccacatacgtggagaaaatgacaccaaaaagggcggtggaaaacttttcaaaggatcacctccacatacgtggagaaaatacttcaactaatcctaattatcctggcaatccaggatcacctccacatacgtggagaaaatgcctagtgccttaccagcctcggcaaaactgtgggatcacctccacatacgtggagaaaatggaacaacgctttctggtga